European Patent Specification EP 4 073 808 B1, published April 15, 2026. Title: Index sequences for multiplex parallel sequencing. Applicant: LEXOGEN GMBH. The sequence listing filed with the application follows.

SEQUENCE LISTING (784 sequences)

SEQ ID NO: 1 - DNA, 12 bp, Artificial Sequence
  index sequence
aaacgttcatcc

SEQ ID NO: 2 - DNA, 12 bp, Artificial Sequence
  index sequence
ttgtccgatatg

SEQ ID NO: 3 - DNA, 12 bp, Artificial Sequence
  index sequence
cgggaacccgca

SEQ ID NO: 4 - DNA, 12 bp, Artificial Sequence
  index sequence
gtttaaaggcag

SEQ ID NO: 5 - DNA, 12 bp, Artificial Sequence
  index sequence
tcctctcttcta

SEQ ID NO: 6 - DNA, 12 bp, Artificial Sequence
  index sequence
ccaaagagggat

SEQ ID NO: 7 - DNA, 12 bp, Artificial Sequence
  index sequence
gaagggtaaagc

SEQ ID NO: 8 - DNA, 12 bp, Artificial Sequence
  index sequence
agtctcagcaaa

SEQ ID NO: 9 - DNA, 12 bp, Artificial Sequence
  index sequence
gcactgacgcta

SEQ ID NO: 10 - DNA, 12 bp, Artificial Sequence
  index sequence
cccaattttgcc

SEQ ID NO: 11 - DNA, 12 bp, Artificial Sequence
  index sequence
cagataatacgt

SEQ ID NO: 12 - DNA, 12 bp, Artificial Sequence
  index sequence
aggtggttctac

SEQ ID NO: 13 - DNA, 12 bp, Artificial Sequence
  index sequence
agaggccgaaca

SEQ ID NO: 14 - DNA, 12 bp, Artificial Sequence
  index sequence
cttaccgggtac

SEQ ID NO: 15 - DNA, 12 bp, Artificial Sequence
  index sequence
tgctaaattagt

SEQ ID NO: 16 - DNA, 12 bp, Artificial Sequence
  index sequence
tacgcccacgtg

SEQ ID NO: 17 - DNA, 12 bp, Artificial Sequence
  index sequence
atcgacttgtgt

SEQ ID NO: 18 - DNA, 12 bp, Artificial Sequence
  index sequence
ctatgcaagctg

SEQ ID NO: 19 - DNA, 12 bp, Artificial Sequence
  index sequence
aaccctgggaag

SEQ ID NO: 20 - DNA, 12 bp, Artificial Sequence
  index sequence
tattggcggcct

SEQ ID NO: 21 - DNA, 12 bp, Artificial Sequence
  index sequence
ccgggcgtcatg

SEQ ID NO: 22 - DNA, 12 bp, Artificial Sequence
  index sequence
gatttcccccga

SEQ ID NO: 23 - DNA, 12 bp, Artificial Sequence
  index sequence
attatatctgaa

SEQ ID NO: 24 - DNA, 12 bp, Artificial Sequence
  index sequence
tcaacaaccggt

SEQ ID NO: 25 - DNA, 12 bp, Artificial Sequence
  index sequence
tggagactgggc

SEQ ID NO: 26 - DNA, 12 bp, Artificial Sequence
  index sequence
ctgtagtcgcca

SEQ ID NO: 27 - DNA, 12 bp, Artificial Sequence
  index sequence
acaggactctgg

SEQ ID NO: 28 - DNA, 12 bp, Artificial Sequence
  index sequence
atttttagggcc

SEQ ID NO: 29 - DNA, 12 bp, Artificial Sequence
  index sequence
ttatcactcctt

SEQ ID NO: 30 - DNA, 12 bp, Artificial Sequence
  index sequence
cactagtttcgt

SEQ ID NO: 31 - DNA, 12 bp, Artificial Sequence
  index sequence
gcctaatacaac

SEQ ID NO: 32 - DNA, 12 bp, Artificial Sequence
  index sequence
acgatacgccaa

SEQ ID NO: 33 - DNA, 12 bp, Artificial Sequence
  index sequence
ccgacggaccat

SEQ ID NO: 34 - DNA, 12 bp, Artificial Sequence
  index sequence
gaattcgtatac

SEQ ID NO: 35 - DNA, 12 bp, Artificial Sequence
  index sequence
gacccgtcttga

SEQ ID NO: 36 - DNA, 12 bp, Artificial Sequence
  index sequence
caccagagatat

SEQ ID NO: 37 - DNA, 12 bp, Artificial Sequence
  index sequence
aaaatcccagtt

SEQ ID NO: 38 - DNA, 12 bp, Artificial Sequence
  index sequence
tacggtatagaa

SEQ ID NO: 39 - DNA, 12 bp, Artificial Sequence
  index sequence
gcatccatgcat

SEQ ID NO: 40 - DNA, 12 bp, Artificial Sequence
  index sequence
gagtcggtggca

SEQ ID NO: 41 - DNA, 12 bp, Artificial Sequence
  index sequence
caccttcggttg

SEQ ID NO: 42 - DNA, 12 bp, Artificial Sequence
  index sequence
ctctttaaacaa

SEQ ID NO: 43 - DNA, 12 bp, Artificial Sequence
  index sequence
gcgtgttaacgc

SEQ ID NO: 44 - DNA, 12 bp, Artificial Sequence
  index sequence
gtgagtagtagt

SEQ ID NO: 45 - DNA, 12 bp, Artificial Sequence
  index sequence
tgccatgttcgg

SEQ ID NO: 46 - DNA, 12 bp, Artificial Sequence
  index sequence
aaatgtagtgag

SEQ ID NO: 47 - DNA, 12 bp, Artificial Sequence
  index sequence
tgtggggtgatt

SEQ ID NO: 48 - DNA, 12 bp, Artificial Sequence
  index sequence
gagcacgcgagc

SEQ ID NO: 49 - DNA, 12 bp, Artificial Sequence
  index sequence
taattacaaaga

SEQ ID NO: 50 - DNA, 12 bp, Artificial Sequence
  index sequence
aagttgcgggta

SEQ ID NO: 51 - DNA, 12 bp, Artificial Sequence
  index sequence
ccgttgaagggg

SEQ ID NO: 52 - DNA, 12 bp, Artificial Sequence
  index sequence
aaactaactgtc

SEQ ID NO: 53 - DNA, 12 bp, Artificial Sequence
  index sequence
gctagctcagat

SEQ ID NO: 54 - DNA, 12 bp, Artificial Sequence
  index sequence
cgagtttatcag

SEQ ID NO: 55 - DNA, 12 bp, Artificial Sequence
  index sequence
agcaaaggatgt

SEQ ID NO: 56 - DNA, 12 bp, Artificial Sequence
  index sequence
tcgagtcccgga

SEQ ID NO: 57 - DNA, 12 bp, Artificial Sequence
  index sequence
ttccaaaaaatg

SEQ ID NO: 58 - DNA, 12 bp, Artificial Sequence
  index sequence
tcctagcgattt

SEQ ID NO: 59 - DNA, 12 bp, Artificial Sequence
  index sequence
taaccagcactt

SEQ ID NO: 60 - DNA, 12 bp, Artificial Sequence
  index sequence
tttgtggacacg

SEQ ID NO: 61 - DNA, 12 bp, Artificial Sequence
  index sequence
ttgcgttctcaa

SEQ ID NO: 62 - DNA, 12 bp, Artificial Sequence
  index sequence
atcggaaaattc

SEQ ID NO: 63 - DNA, 12 bp, Artificial Sequence
  index sequence
actaagcgcgtg

SEQ ID NO: 64 - DNA, 12 bp, Artificial Sequence
  index sequence
ccgccctatttc

SEQ ID NO: 65 - DNA, 12 bp, Artificial Sequence
  index sequence
cttaatgatatc

SEQ ID NO: 66 - DNA, 12 bp, Artificial Sequence
  index sequence
tgttttgctaac

SEQ ID NO: 67 - DNA, 12 bp, Artificial Sequence
  index sequence
gaaaatttacgc

SEQ ID NO: 68 - DNA, 12 bp, Artificial Sequence
  index sequence
ttgacagcgtcg

SEQ ID NO: 69 - DNA, 12 bp, Artificial Sequence
  index sequence
cctggtactttc

SEQ ID NO: 70 - DNA, 12 bp, Artificial Sequence
  index sequence
gtcaggctgcgt

SEQ ID NO: 71 - DNA, 12 bp, Artificial Sequence
  index sequence
ctctccatcgaa

SEQ ID NO: 72 - DNA, 12 bp, Artificial Sequence
  index sequence
gcgccgggtccc

SEQ ID NO: 73 - DNA, 12 bp, Artificial Sequence
  index sequence
tataagggaatg

SEQ ID NO: 74 - DNA, 12 bp, Artificial Sequence
  index sequence
attcctgagtta

SEQ ID NO: 75 - DNA, 12 bp, Artificial Sequence
  index sequence
cccaccgtaagc

SEQ ID NO: 76 - DNA, 12 bp, Artificial Sequence
  index sequence
aatagctttttc

SEQ ID NO: 77 - DNA, 12 bp, Artificial Sequence
  index sequence
gtaccgaacccg

SEQ ID NO: 78 - DNA, 12 bp, Artificial Sequence
  index sequence
ttccccgtttag

SEQ ID NO: 79 - DNA, 12 bp, Artificial Sequence
  index sequence
acccgaacgagc

SEQ ID NO: 80 - DNA, 12 bp, Artificial Sequence
  index sequence
aagccacccccg

SEQ ID NO: 81 - DNA, 12 bp, Artificial Sequence
  index sequence
atgcattgccct

SEQ ID NO: 82 - DNA, 12 bp, Artificial Sequence
  index sequence
aggcttaatcgg

SEQ ID NO: 83 - DNA, 12 bp, Artificial Sequence
  index sequence
ttaggacgcaaa

SEQ ID NO: 84 - DNA, 12 bp, Artificial Sequence
  index sequence
cgaccactaccg

SEQ ID NO: 85 - DNA, 12 bp, Artificial Sequence
  index sequence
cgggtagggcgt

SEQ ID NO: 86 - DNA, 12 bp, Artificial Sequence
  index sequence
aatgaccgtagg

SEQ ID NO: 87 - DNA, 12 bp, Artificial Sequence
  index sequence
attcaacctcta

SEQ ID NO: 88 - DNA, 12 bp, Artificial Sequence
  index sequence
caaggtcccctt

SEQ ID NO: 89 - DNA, 12 bp, Artificial Sequence
  index sequence
gatagaaacacc

SEQ ID NO: 90 - DNA, 12 bp, Artificial Sequence
  index sequence
gtggcaccactt

SEQ ID NO: 91 - DNA, 12 bp, Artificial Sequence
  index sequence
agcttcttttcc

SEQ ID NO: 92 - DNA, 12 bp, Artificial Sequence
  index sequence
tcgtctggccgt

SEQ ID NO: 93 - DNA, 12 bp, Artificial Sequence
  index sequence
atccgccaggat

SEQ ID NO: 94 - DNA, 12 bp, Artificial Sequence
  index sequence
tgaggcatttgg

SEQ ID NO: 95 - DNA, 12 bp, Artificial Sequence
  index sequence
gacattattctt

SEQ ID NO: 96 - DNA, 12 bp, Artificial Sequence
  index sequence
taagatcgatta

SEQ ID NO: 97 - DNA, 12 bp, Artificial Sequence
  index sequence
gtttgactttat

SEQ ID NO: 98 - DNA, 12 bp, Artificial Sequence
  index sequence
aaaacatgcgtt

SEQ ID NO: 99 - DNA, 12 bp, Artificial Sequence
  index sequence
caaattggaacg

SEQ ID NO: 100 - DNA, 12 bp, Artificial Sequence
  index sequence
atgggctagaca

SEQ ID NO: 101 - DNA, 12 bp, Artificial Sequence
  index sequence
gcgcgaagttga

SEQ ID NO: 102 - DNA, 12 bp, Artificial Sequence
  index sequence
ccattgtctaaa

SEQ ID NO: 103 - DNA, 12 bp, Artificial Sequence
  index sequence
tcccggctaaaa

SEQ ID NO: 104 - DNA, 12 bp, Artificial Sequence
  index sequence
gtcaaatgtcct

SEQ ID NO: 105 - DNA, 12 bp, Artificial Sequence
  index sequence
cccagttactaa

SEQ ID NO: 106 - DNA, 12 bp, Artificial Sequence
  index sequence
ttgtaagctctg

SEQ ID NO: 107 - DNA, 12 bp, Artificial Sequence
  index sequence
agggccaaagac

SEQ ID NO: 108 - DNA, 12 bp, Artificial Sequence
  index sequence
gtttcccggacg

SEQ ID NO: 109 - DNA, 12 bp, Artificial Sequence
  index sequence
taatatattatc

SEQ ID NO: 110 - DNA, 12 bp, Artificial Sequence
  index sequence
aacccgcgggct

SEQ ID NO: 111 - DNA, 12 bp, Artificial Sequence
  index sequence
gccgggtcccga

SEQ ID NO: 112 - DNA, 12 bp, Artificial Sequence
  index sequence
cgtatacgaccc

SEQ ID NO: 113 - DNA, 12 bp, Artificial Sequence
  index sequence
gacatgcagatc

SEQ ID NO: 114 - DNA, 12 bp, Artificial Sequence
  index sequence
aaaccttttgaa

SEQ ID NO: 115 - DNA, 12 bp, Artificial Sequence
  index sequence
acgctcctcagt

SEQ ID NO: 116 - DNA, 12 bp, Artificial Sequence
  index sequence
cggtggttatca

SEQ ID NO: 117 - DNA, 12 bp, Artificial Sequence
  index sequence
cgcggaagccac

SEQ ID NO: 118 - DNA, 12 bp, Artificial Sequence
  index sequence
attcaagggtca

SEQ ID NO: 119 - DNA, 12 bp, Artificial Sequence
  index sequence
tgatcccttcgt

SEQ ID NO: 120 - DNA, 12 bp, Artificial Sequence
  index sequence
tcagaaacagtg

SEQ ID NO: 121 - DNA, 12 bp, Artificial Sequence
  index sequence
ctagcattgtgt

SEQ ID NO: 122 - DNA, 12 bp, Artificial Sequence
  index sequence
atctgaccgatg

SEQ ID NO: 123 - DNA, 12 bp, Artificial Sequence
  index sequence
ccaaatgggccg

SEQ ID NO: 124 - DNA, 12 bp, Artificial Sequence
  index sequence
tcttggaggaat

SEQ ID NO: 125 - DNA, 12 bp, Artificial Sequence
  index sequence
aagggagtactg

SEQ ID NO: 126 - DNA, 12 bp, Artificial Sequence
  index sequence
gctttaaaaagc

SEQ ID NO: 127 - DNA, 12 bp, Artificial Sequence
  index sequence
cttctctatgcc

SEQ ID NO: 128 - DNA, 12 bp, Artificial Sequence
  index sequence
taccaccaaggt

SEQ ID NO: 129 - DNA, 12 bp, Artificial Sequence
  index sequence
tggcgcatggga

SEQ ID NO: 130 - DNA, 12 bp, Artificial Sequence
  index sequence
atgtcgtagaac

SEQ ID NO: 131 - DNA, 12 bp, Artificial Sequence
  index sequence
cacggcatatgg

SEQ ID NO: 132 - DNA, 12 bp, Artificial Sequence
  index sequence
ctttttcgggaa

SEQ ID NO: 133 - DNA, 12 bp, Artificial Sequence
  index sequence
ttctacataatt

SEQ ID NO: 134 - DNA, 12 bp, Artificial Sequence
  index sequence
acatcgtttagt

SEQ ID NO: 135 - DNA, 12 bp, Artificial Sequence
  index sequence
gaatcctcacca

SEQ ID NO: 136 - DNA, 12 bp, Artificial Sequence
  index sequence
cagctcagaacc

SEQ ID NO: 137 - DNA, 12 bp, Artificial Sequence
  index sequence
aagcaggcaact

SEQ ID NO: 138 - DNA, 12 bp, Artificial Sequence
  index sequence
gccttagtctca

SEQ ID NO: 139 - DNA, 12 bp, Artificial Sequence
  index sequence
gcaaagtattgc

SEQ ID NO: 140 - DNA, 12 bp, Artificial Sequence
  index sequence
acaacgcgctct

SEQ ID NO: 141 - DNA, 12 bp, Artificial Sequence
  index sequence
cccctaaacgtt

SEQ ID NO: 142 - DNA, 12 bp, Artificial Sequence
  index sequence
tcaggtctcgcc

SEQ ID NO: 143 - DNA, 12 bp, Artificial Sequence
  index sequence
gactaactgact

SEQ ID NO: 144 - DNA, 12 bp, Artificial Sequence
  index sequence
gcgtaggtggac

SEQ ID NO: 145 - DNA, 12 bp, Artificial Sequence
  index sequence
acaattaggttg

SEQ ID NO: 146 - DNA, 12 bp, Artificial Sequence
  index sequence
atatttcccacc

SEQ ID NO: 147 - DNA, 12 bp, Artificial Sequence
  index sequence
gagtgttccaga

SEQ ID NO: 148 - DNA, 12 bp, Artificial Sequence
  index sequence
gtgcgtcgtcgt

SEQ ID NO: 149 - DNA, 12 bp, Artificial Sequence
  index sequence
tgaactgttagg

SEQ ID NO: 150 - DNA, 12 bp, Artificial Sequence
  index sequence
ccctgtcgtgcg

SEQ ID NO: 151 - DNA, 12 bp, Artificial Sequence
  index sequence
tgtggggtgctt

SEQ ID NO: 152 - DNA, 12 bp, Artificial Sequence
  index sequence
gcgacagagcga

SEQ ID NO: 153 - DNA, 12 bp, Artificial Sequence
  index sequence
tccttcacccgc

SEQ ID NO: 154 - DNA, 12 bp, Artificial Sequence
  index sequence
ccgttgagggtc

SEQ ID NO: 155 - DNA, 12 bp, Artificial Sequence
  index sequence
aagttgccgggg

SEQ ID NO: 156 - DNA, 12 bp, Artificial Sequence
  index sequence
cccatccatgta

SEQ ID NO: 157 - DNA, 12 bp, Artificial Sequence
  index sequence
gatcgatacgct

SEQ ID NO: 158 - DNA, 12 bp, Artificial Sequence
  index sequence
agcgtttctacg

SEQ ID NO: 159 - DNA, 12 bp, Artificial Sequence
  index sequence
cgacccggctgt

SEQ ID NO: 160 - DNA, 12 bp, Artificial Sequence
  index sequence
tagcgtaaaggc

SEQ ID NO: 161 - DNA, 12 bp, Artificial Sequence
  index sequence
ttaacccccctg

SEQ ID NO: 162 - DNA, 12 bp, Artificial Sequence
  index sequence
taatcgagcttt

SEQ ID NO: 163 - DNA, 12 bp, Artificial Sequence
  index sequence
tccaacgacatt

SEQ ID NO: 164 - DNA, 12 bp, Artificial Sequence
  index sequence
tttgtggcacag

SEQ ID NO: 165 - DNA, 12 bp, Artificial Sequence
  index sequence
ttgagttatacc

SEQ ID NO: 166 - DNA, 12 bp, Artificial Sequence
  index sequence
ctaggcccctta

SEQ ID NO: 167 - DNA, 12 bp, Artificial Sequence
  index sequence
catccgagagtg

SEQ ID NO: 168 - DNA, 12 bp, Artificial Sequence
  index sequence
aagaaatcttta

SEQ ID NO: 169 - DNA, 12 bp, Artificial Sequence
  index sequence
attcctgctcta

SEQ ID NO: 170 - DNA, 12 bp, Artificial Sequence
  index sequence
tgttttgatcca

SEQ ID NO: 171 - DNA, 12 bp, Artificial Sequence
  index sequence
gcccctttcaga

SEQ ID NO: 172 - DNA, 12 bp, Artificial Sequence
  index sequence
ttgcacgagtag

SEQ ID NO: 173 - DNA, 12 bp, Artificial Sequence
  index sequence
aatggtcattta

SEQ ID NO: 174 - DNA, 12 bp, Artificial Sequence
  index sequence
gtacggatgagt

SEQ ID NO: 175 - DNA, 12 bp, Artificial Sequence
  index sequence
atataactagcc

SEQ ID NO: 176 - DNA, 12 bp, Artificial Sequence
  index sequence
gagaagggtaaa

SEQ ID NO: 177 - DNA, 12 bp, Artificial Sequence
  index sequence
tctccgggcctg

SEQ ID NO: 178 - DNA, 12 bp, Artificial Sequence
  index sequence
cttaatgcgttc

SEQ ID NO: 179 - DNA, 12 bp, Artificial Sequence
  index sequence
aaacaagtccga

SEQ ID NO: 180 - DNA, 12 bp, Artificial Sequence
  index sequence
cctcgattttta

SEQ ID NO: 181 - DNA, 12 bp, Artificial Sequence
  index sequence
gtcaagccaaag

SEQ ID NO: 182 - DNA, 12 bp, Artificial Sequence
  index sequence
ttaaaagtttcg

SEQ ID NO: 183 - DNA, 12 bp, Artificial Sequence
  index sequence
caaagccagcga

SEQ ID NO: 184 - DNA, 12 bp, Artificial Sequence
  index sequence
ccgaacaaaaag

SEQ ID NO: 185 - DNA, 12 bp, Artificial Sequence
  index sequence
ctgacttgaaat

SEQ ID NO: 186 - DNA, 12 bp, Artificial Sequence
  index sequence
cggattcctagg

SEQ ID NO: 187 - DNA, 12 bp, Artificial Sequence
  index sequence
ttcggcagaccc

SEQ ID NO: 188 - DNA, 12 bp, Artificial Sequence
  index sequence
agcaacatcaag

SEQ ID NO: 189 - DNA, 12 bp, Artificial Sequence
  index sequence
agggtcgggagt

SEQ ID NO: 190 - DNA, 12 bp, Artificial Sequence
  index sequence
cctgcaagtcgg

SEQ ID NO: 191 - DNA, 12 bp, Artificial Sequence
  index sequence
cttaccaatatc

SEQ ID NO: 192 - DNA, 12 bp, Artificial Sequence
  index sequence
accggtaaaatt

SEQ ID NO: 193 - DNA, 12 bp, Artificial Sequence
  index sequence
gctcgcccacaa

SEQ ID NO: 194 - DNA, 12 bp, Artificial Sequence
  index sequence
gtggacaacatt

SEQ ID NO: 195 - DNA, 12 bp, Artificial Sequence
  index sequence
cgattattttaa

SEQ ID NO: 196 - DNA, 12 bp, Artificial Sequence
  index sequence
tagtatggaagt

SEQ ID NO: 197 - DNA, 12 bp, Artificial Sequence
  index sequence
ctaagaacggct

SEQ ID NO: 198 - DNA, 12 bp, Artificial Sequence
  index sequence
tgcggactttgg

SEQ ID NO: 199 - DNA, 12 bp, Artificial Sequence
  index sequence
gcacttcttatt

SEQ ID NO: 200 - DNA, 12 bp, Artificial Sequence
  index sequence
tccgctagcttc

SEQ ID NO: 201 - DNA, 12 bp, Artificial Sequence
  index sequence
gtttgcatttct

SEQ ID NO: 202 - DNA, 12 bp, Artificial Sequence
  index sequence
ccccactgagtt

SEQ ID NO: 203 - DNA, 12 bp, Artificial Sequence
  index sequence
acccttggccag

SEQ ID NO: 204 - DNA, 12 bp, Artificial Sequence
  index sequence
ctgggatcgcac

SEQ ID NO: 205 - DNA, 12 bp, Artificial Sequence
  index sequence
gagagccgttgc

SEQ ID NO: 206 - DNA, 12 bp, Artificial Sequence
  index sequence
aacttgtatccc

SEQ ID NO: 207 - DNA, 12 bp, Artificial Sequence
  index sequence
taaaggatcccc

SEQ ID NO: 208 - DNA, 12 bp, Artificial Sequence
  index sequence
gtaccctgtaat

SEQ ID NO: 209 - DNA, 12 bp, Artificial Sequence
  index sequence
agtattatgccc

SEQ ID NO: 210 - DNA, 12 bp, Artificial Sequence
  index sequence
agcacacttaca

SEQ ID NO: 211 - DNA, 12 bp, Artificial Sequence
  index sequence
agaatgtcgaca

SEQ ID NO: 212 - DNA, 12 bp, Artificial Sequence
  index sequence
aagtaacagctt

SEQ ID NO: 213 - DNA, 12 bp, Artificial Sequence
  index sequence
tagactctgact

SEQ ID NO: 214 - DNA, 12 bp, Artificial Sequence
  index sequence
atagacgatccc

SEQ ID NO: 215 - DNA, 12 bp, Artificial Sequence
  index sequence
tcatgccgaact

SEQ ID NO: 216 - DNA, 12 bp, Artificial Sequence
  index sequence
cgtcgaatatgg

SEQ ID NO: 217 - DNA, 12 bp, Artificial Sequence
  index sequence
atgacccagatg

SEQ ID NO: 218 - DNA, 12 bp, Artificial Sequence
  index sequence
atttggccgatt

SEQ ID NO: 219 - DNA, 12 bp, Artificial Sequence
  index sequence
agtggcgcaagc

SEQ ID NO: 220 - DNA, 12 bp, Artificial Sequence
  index sequence
cgccttttaggg

SEQ ID NO: 221 - DNA, 12 bp, Artificial Sequence
  index sequence
ctcggtgatcgt

SEQ ID NO: 222 - DNA, 12 bp, Artificial Sequence
  index sequence
ccgtgtgctgaa

SEQ ID NO: 223 - DNA, 12 bp, Artificial Sequence
  index sequence
atcctgtgccta

SEQ ID NO: 224 - DNA, 12 bp, Artificial Sequence
  index sequence
tctaatctgacg

SEQ ID NO: 225 - DNA, 12 bp, Artificial Sequence
  index sequence
agtggataagtt

SEQ ID NO: 226 - DNA, 12 bp, Artificial Sequence
  index sequence
tgccctcaaacc

SEQ ID NO: 227 - DNA, 12 bp, Artificial Sequence
  index sequence
ctcccctgtgac

SEQ ID NO: 228 - DNA, 12 bp, Artificial Sequence
  index sequence
gtatgcggtagc

SEQ ID NO: 229 - DNA, 12 bp, Artificial Sequence
  index sequence
ccactacatctt

SEQ ID NO: 230 - DNA, 12 bp, Artificial Sequence
  index sequence
ctaaacttcttg

SEQ ID NO: 231 - DNA, 12 bp, Artificial Sequence
  index sequence
gcagatatggta

SEQ ID NO: 232 - DNA, 12 bp, Artificial Sequence
  index sequence
tctgcttgaggt

SEQ ID NO: 233 - DNA, 12 bp, Artificial Sequence
  index sequence
gaaatgtgaagg

SEQ ID NO: 234 - DNA, 12 bp, Artificial Sequence
  index sequence
caaacgctgagg

SEQ ID NO: 235 - DNA, 12 bp, Artificial Sequence
  index sequence
gctactttgggg

SEQ ID NO: 236 - DNA, 12 bp, Artificial Sequence
  index sequence
agaaattggcat

SEQ ID NO: 237 - DNA, 12 bp, Artificial Sequence
  index sequence
ctgccaacacga

SEQ ID NO: 238 - DNA, 12 bp, Artificial Sequence
  index sequence
ccaaatccttcg

SEQ ID NO: 239 - DNA, 12 bp, Artificial Sequence
  index sequence
cgcccaaatatc

SEQ ID NO: 240 - DNA, 12 bp, Artificial Sequence
  index sequence
tttatcgttaat

SEQ ID NO: 241 - DNA, 12 bp, Artificial Sequence
  index sequence
acgtcaacgtcc

SEQ ID NO: 242 - DNA, 12 bp, Artificial Sequence
  index sequence
tcaggtaaactt

SEQ ID NO: 243 - DNA, 12 bp, Artificial Sequence
  index sequence
agagtattagag

SEQ ID NO: 244 - DNA, 12 bp, Artificial Sequence
  index sequence
tacatggccact

SEQ ID NO: 245 - DNA, 12 bp, Artificial Sequence
  index sequence
gcaggttctcgt

SEQ ID NO: 246 - DNA, 12 bp, Artificial Sequence
  index sequence
cgatgataacgg

SEQ ID NO: 247 - DNA, 12 bp, Artificial Sequence
  index sequence
agttctacggac

SEQ ID NO: 248 - DNA, 12 bp, Artificial Sequence
  index sequence
tctcagattcat

SEQ ID NO: 249 - DNA, 12 bp, Artificial Sequence
  index sequence
actgtcccgcta

SEQ ID NO: 250 - DNA, 12 bp, Artificial Sequence
  index sequence
atgacggtgagc

SEQ ID NO: 251 - DNA, 12 bp, Artificial Sequence
  index sequence
gaccgtgcgcaa

SEQ ID NO: 252 - DNA, 12 bp, Artificial Sequence
  index sequence
tactcgtgctgt

SEQ ID NO: 253 - DNA, 12 bp, Artificial Sequence
  index sequence
gttcataatcac

SEQ ID NO: 254 - DNA, 12 bp, Artificial Sequence
  index sequence
agagaagcgtta

SEQ ID NO: 255 - DNA, 12 bp, Artificial Sequence
  index sequence
aggacatcggac

SEQ ID NO: 256 - DNA, 12 bp, Artificial Sequence
  index sequence
tgcgttaactct

SEQ ID NO: 257 - DNA, 12 bp, Artificial Sequence
  index sequence
aacttgtaaata

SEQ ID NO: 258 - DNA, 12 bp, Artificial Sequence
  index sequence
tatcctactcat

SEQ ID NO: 259 - DNA, 12 bp, Artificial Sequence
  index sequence
ccacgagcactg

SEQ ID NO: 260 - DNA, 12 bp, Artificial Sequence
  index sequence
gcgttcgatgaa

SEQ ID NO: 261 - DNA, 12 bp, Artificial Sequence
  index sequence
ttagctatcttg

SEQ ID NO: 262 - DNA, 12 bp, Artificial Sequence
  index sequence
aggtcctgggga

SEQ ID NO: 263 - DNA, 12 bp, Artificial Sequence
  index sequence
acttcgtccagt

SEQ ID NO: 264 - DNA, 12 bp, Artificial Sequence
  index sequence
tagtgcttctaa

SEQ ID NO: 265 - DNA, 12 bp, Artificial Sequence
  index sequence
gccggaggtctg

SEQ ID NO: 266 - DNA, 12 bp, Artificial Sequence
  index sequence
gttcgatcagta

SEQ ID NO: 267 - DNA, 12 bp, Artificial Sequence
  index sequence
ccagaagttatt

SEQ ID NO: 268 - DNA, 12 bp, Artificial Sequence
  index sequence
catagggagggg

SEQ ID NO: 269 - DNA, 12 bp, Artificial Sequence
  index sequence
caggcgcgaaga

SEQ ID NO: 270 - DNA, 12 bp, Artificial Sequence
  index sequence
cccgatagtaca

SEQ ID NO: 271 - DNA, 12 bp, Artificial Sequence
  index sequence
agcccgcgtcgt

SEQ ID NO: 272 - DNA, 12 bp, Artificial Sequence
  index sequence
tggccatacgta

SEQ ID NO: 273 - DNA, 12 bp, Artificial Sequence
  index sequence
aagcggcagagg

SEQ ID NO: 274 - DNA, 12 bp, Artificial Sequence
  index sequence
tacgcagtacaa

SEQ ID NO: 275 - DNA, 12 bp, Artificial Sequence
  index sequence
tctgtaattgca

SEQ ID NO: 276 - DNA, 12 bp, Artificial Sequence
  index sequence
taccattcgcag

SEQ ID NO: 277 - DNA, 12 bp, Artificial Sequence
  index sequence
cgcaagccctcg

SEQ ID NO: 278 - DNA, 12 bp, Artificial Sequence
  index sequence
cacgcgatgggc

SEQ ID NO: 279 - DNA, 12 bp, Artificial Sequence
  index sequence
cacacaagggag

SEQ ID NO: 280 - DNA, 12 bp, Artificial Sequence
  index sequence
ttagtgttaaaa

SEQ ID NO: 281 - DNA, 12 bp, Artificial Sequence
  index sequence
taggggacatca

SEQ ID NO: 282 - DNA, 12 bp, Artificial Sequence
  index sequence
gaaagatcgccg

SEQ ID NO: 283 - DNA, 12 bp, Artificial Sequence
  index sequence
gaacgagaatgt

SEQ ID NO: 284 - DNA, 12 bp, Artificial Sequence
  index sequence
gcctcctccgtg

SEQ ID NO: 285 - DNA, 12 bp, Artificial Sequence
  index sequence
ctgatgtgagag

SEQ ID NO: 286 - DNA, 12 bp, Artificial Sequence
  index sequence
attgatcaagct

SEQ ID NO: 287 - DNA, 12 bp, Artificial Sequence
  index sequence
agacgggcacaa

SEQ ID NO: 288 - DNA, 12 bp, Artificial Sequence
  index sequence
ccctgcttacga

SEQ ID NO: 289 - DNA, 12 bp, Artificial Sequence
  index sequence
ttaatgcgtgat

SEQ ID NO: 290 - DNA, 12 bp, Artificial Sequence
  index sequence
gtgctaatggga

SEQ ID NO: 291 - DNA, 12 bp, Artificial Sequence
  index sequence
cttaacacataa

SEQ ID NO: 292 - DNA, 12 bp, Artificial Sequence
  index sequence
aaaaacggcagg

SEQ ID NO: 293 - DNA, 12 bp, Artificial Sequence
  index sequence
tgtttgagtcgg

SEQ ID NO: 294 - DNA, 12 bp, Artificial Sequence
  index sequence
tgcccgacaggt

SEQ ID NO: 295 - DNA, 12 bp, Artificial Sequence
  index sequence
aacgaatctgta

SEQ ID NO: 296 - DNA, 12 bp, Artificial Sequence
  index sequence
gtcatccgtttt

SEQ ID NO: 297 - DNA, 12 bp, Artificial Sequence
  index sequence
ataactctcctc

SEQ ID NO: 298 - DNA, 12 bp, Artificial Sequence
  index sequence
tagaatacggtt

SEQ ID NO: 299 - DNA, 12 bp, Artificial Sequence
  index sequence
acgttttgattc

SEQ ID NO: 300 - DNA, 12 bp, Artificial Sequence
  index sequence
cgacctgaacgg

SEQ ID NO: 301 - DNA, 12 bp, Artificial Sequence
  index sequence
agtgtgaccggt

SEQ ID NO: 302 - DNA, 12 bp, Artificial Sequence
  index sequence
ttataagccgtc

SEQ ID NO: 303 - DNA, 12 bp, Artificial Sequence
  index sequence
tattgaactcca

SEQ ID NO: 304 - DNA, 12 bp, Artificial Sequence
  index sequence
cagttcctaacc

SEQ ID NO: 305 - DNA, 12 bp, Artificial Sequence
  index sequence
acattcaagtgc

SEQ ID NO: 306 - DNA, 12 bp, Artificial Sequence
  index sequence
gcgacgctcgta

SEQ ID NO: 307 - DNA, 12 bp, Artificial Sequence
  index sequence
cgtgatttaaag

SEQ ID NO: 308 - DNA, 12 bp, Artificial Sequence
  index sequence
acctacagacct

SEQ ID NO: 309 - DNA, 12 bp, Artificial Sequence
  index sequence
gtttattcagtg

SEQ ID NO: 310 - DNA, 12 bp, Artificial Sequence
  index sequence
gctcaccctctt

SEQ ID NO: 311 - DNA, 12 bp, Artificial Sequence
  index sequence
acctgatgtatt

SEQ ID NO: 312 - DNA, 12 bp, Artificial Sequence
  index sequence
agttatgtgcag

SEQ ID NO: 313 - DNA, 12 bp, Artificial Sequence
  index sequence
tcggctcacaag

SEQ ID NO: 314 - DNA, 12 bp, Artificial Sequence
  index sequence
gctgcatacaag

SEQ ID NO: 315 - DNA, 12 bp, Artificial Sequence
  index sequence
gccccacatgat

SEQ ID NO: 316 - DNA, 12 bp, Artificial Sequence
  index sequence
aaagcctatcac

SEQ ID NO: 317 - DNA, 12 bp, Artificial Sequence
  index sequence
ctatgtttttgc

SEQ ID NO: 318 - DNA, 12 bp, Artificial Sequence
  index sequence
cacgggtcagaa

SEQ ID NO: 319 - DNA, 12 bp, Artificial Sequence
  index sequence
gcgtaggcaaga

SEQ ID NO: 320 - DNA, 12 bp, Artificial Sequence
  index sequence
tgtcgcaacggc

SEQ ID NO: 321 - DNA, 12 bp, Artificial Sequence
  index sequence
atctcattatgg

SEQ ID NO: 322 - DNA, 12 bp, Artificial Sequence
  index sequence
gagatcagtcag

SEQ ID NO: 323 - DNA, 12 bp, Artificial Sequence
  index sequence
ttcgaaccgaga

SEQ ID NO: 324 - DNA, 12 bp, Artificial Sequence
  index sequence
ctcactccgccc

SEQ ID NO: 325 - DNA, 12 bp, Artificial Sequence
  index sequence
tttgcaaagccg

SEQ ID NO: 326 - DNA, 12 bp, Artificial Sequence
  index sequence
cttgtaacgagt

SEQ ID NO: 327 - DNA, 12 bp, Artificial Sequence
  index sequence
gagtgtctgagg

SEQ ID NO: 328 - DNA, 12 bp, Artificial Sequence
  index sequence
acggcgccaggg

SEQ ID NO: 329 - DNA, 12 bp, Artificial Sequence
  index sequence
gtaagcacgtat

SEQ ID NO: 330 - DNA, 12 bp, Artificial Sequence
  index sequence
aagtctttgtcg

SEQ ID NO: 331 - DNA, 12 bp, Artificial Sequence
  index sequence
gacttcaatcga

SEQ ID NO: 332 - DNA, 12 bp, Artificial Sequence
  index sequence
tctagacaaagt

SEQ ID NO: 333 - DNA, 12 bp, Artificial Sequence
  index sequence
gatgcgctcctt

SEQ ID NO: 334 - DNA, 12 bp, Artificial Sequence
  index sequence
gtactcccaatg

SEQ ID NO: 335 - DNA, 12 bp, Artificial Sequence
  index sequence
tagcgaatatct

SEQ ID NO: 336 - DNA, 12 bp, Artificial Sequence
  index sequence
gcattgcgaatt

SEQ ID NO: 337 - DNA, 12 bp, Artificial Sequence
  index sequence
atggctggctca

SEQ ID NO: 338 - DNA, 12 bp, Artificial Sequence
  index sequence
tatcaatacccg

SEQ ID NO: 339 - DNA, 12 bp, Artificial Sequence
  index sequence
tcataaaggcca

SEQ ID NO: 340 - DNA, 12 bp, Artificial Sequence
  index sequence
tgtgccctataa

SEQ ID NO: 341 - DNA, 12 bp, Artificial Sequence
  index sequence
aggcaagaacgt

SEQ ID NO: 342 - DNA, 12 bp, Artificial Sequence
  index sequence
gtgcggccgagt

SEQ ID NO: 343 - DNA, 12 bp, Artificial Sequence
  index sequence
gcggagcaccca

SEQ ID NO: 344 - DNA, 12 bp, Artificial Sequence
  index sequence
cgctcggtggga

SEQ ID NO: 345 - DNA, 12 bp, Artificial Sequence
  index sequence
accctagatcgc

SEQ ID NO: 346 - DNA, 12 bp, Artificial Sequence
  index sequence
cagaacgaatcc

SEQ ID NO: 347 - DNA, 12 bp, Artificial Sequence
  index sequence
ccgcaatgaact

SEQ ID NO: 348 - DNA, 12 bp, Artificial Sequence
  index sequence
tgagaggggttc

SEQ ID NO: 349 - DNA, 12 bp, Artificial Sequence
  index sequence
catacttatttg

SEQ ID NO: 350 - DNA, 12 bp, Artificial Sequence
  index sequence
catcgacgtacg

SEQ ID NO: 351 - DNA, 12 bp, Artificial Sequence
  index sequence
gccatctataga

SEQ ID NO: 352 - DNA, 12 bp, Artificial Sequence
  index sequence
gcctctgaacta

SEQ ID NO: 353 - DNA, 12 bp, Artificial Sequence
  index sequence
cccaggcagctt

SEQ ID NO: 354 - DNA, 12 bp, Artificial Sequence
  index sequence
tagcccggggca

SEQ ID NO: 355 - DNA, 12 bp, Artificial Sequence
  index sequence
cacgtaccagtc

SEQ ID NO: 356 - DNA, 12 bp, Artificial Sequence
  index sequence
aatccggcgcac

SEQ ID NO: 357 - DNA, 12 bp, Artificial Sequence
  index sequence
cctctcgacatt

SEQ ID NO: 358 - DNA, 12 bp, Artificial Sequence
  index sequence
actgcgatcgtc

SEQ ID NO: 359 - DNA, 12 bp, Artificial Sequence
  index sequence
gtccaactcaaa

SEQ ID NO: 360 - DNA, 12 bp, Artificial Sequence
  index sequence
tttcttcctcgc

SEQ ID NO: 361 - DNA, 12 bp, Artificial Sequence
  index sequence
tagccgttgtac

SEQ ID NO: 362 - DNA, 12 bp, Artificial Sequence
  index sequence
gacgatcctcac

SEQ ID NO: 363 - DNA, 12 bp, Artificial Sequence
  index sequence
gtgcttgcaaac

SEQ ID NO: 364 - DNA, 12 bp, Artificial Sequence
  index sequence
cagtgaggtact

SEQ ID NO: 365 - DNA, 12 bp, Artificial Sequence
  index sequence
tagtttagggtg

SEQ ID NO: 366 - DNA, 12 bp, Artificial Sequence
  index sequence
ttttcgggatgg

SEQ ID NO: 367 - DNA, 12 bp, Artificial Sequence
  index sequence
gattacatgaga

SEQ ID NO: 368 - DNA, 12 bp, Artificial Sequence
  index sequence
ttcaacggtaag

SEQ ID NO: 369 - DNA, 12 bp, Artificial Sequence
  index sequence
aaggtagatgcg

SEQ ID NO: 370 - DNA, 12 bp, Artificial Sequence
  index sequence
ttcacgaatgct

SEQ ID NO: 371 - DNA, 12 bp, Artificial Sequence
  index sequence
attcccttggta

SEQ ID NO: 372 - DNA, 12 bp, Artificial Sequence
  index sequence
agctccgatgcc

SEQ ID NO: 373 - DNA, 12 bp, Artificial Sequence
  index sequence
cgcaactagaag

SEQ ID NO: 374 - DNA, 12 bp, Artificial Sequence
  index sequence
tatggttaccag

SEQ ID NO: 375 - DNA, 12 bp, Artificial Sequence
  index sequence
gctacgagagag

SEQ ID NO: 376 - DNA, 12 bp, Artificial Sequence
  index sequence
tggcggcggcga

SEQ ID NO: 377 - DNA, 12 bp, Artificial Sequence
  index sequence
agatggcaaccc

SEQ ID NO: 378 - DNA, 12 bp, Artificial Sequence
  index sequence
agtaaccacagc

SEQ ID NO: 379 - DNA, 12 bp, Artificial Sequence
  index sequence
ccttttgtaccc

SEQ ID NO: 380 - DNA, 12 bp, Artificial Sequence
  index sequence
ataagaagtgcc

SEQ ID NO: 381 - DNA, 12 bp, Artificial Sequence
  index sequence
aatcggagtaga

SEQ ID NO: 382 - DNA, 12 bp, Artificial Sequence
  index sequence
gcagtaagctgt

SEQ ID NO: 383 - DNA, 12 bp, Artificial Sequence
  index sequence
cgcggcacgata

SEQ ID NO: 384 - DNA, 12 bp, Artificial Sequence
  index sequence
ctgcagctactt

SEQ ID NO: 385 - DNA, 12 bp, Artificial Sequence
  index sequence
acagggggtgtc

SEQ ID NO: 386 - DNA, 12 bp, Artificial Sequence
  index sequence
gatccaagaggg

SEQ ID NO: 387 - DNA, 12 bp, Artificial Sequence
  index sequence
gacagtcgagag

SEQ ID NO: 388 - DNA, 12 bp, Artificial Sequence
  index sequence
gttggagaaata

SEQ ID NO: 389 - DNA, 12 bp, Artificial Sequence
  index sequence
tcactctaggat

SEQ ID NO: 390 - DNA, 12 bp, Artificial Sequence
  index sequence
ttaataaacgta

SEQ ID NO: 391 - DNA, 12 bp, Artificial Sequence
  index sequence
ttgatattcgca

SEQ ID NO: 392 - DNA, 12 bp, Artificial Sequence
  index sequence
cgttggctcgcg

SEQ ID NO: 393 - DNA, 12 bp, Artificial Sequence
  index sequence
cgtctgtcttca

SEQ ID NO: 394 - DNA, 12 bp, Artificial Sequence
  index sequence
aacagtgtcacc

SEQ ID NO: 395 - DNA, 12 bp, Artificial Sequence
  index sequence
gcgattaaatca

SEQ ID NO: 396 - DNA, 12 bp, Artificial Sequence
  index sequence
cggagccgaccg

SEQ ID NO: 397 - DNA, 12 bp, Artificial Sequence
  index sequence
gtatagttgcga

SEQ ID NO: 398 - DNA, 12 bp, Artificial Sequence
  index sequence
cgagcatcgggt

SEQ ID NO: 399 - DNA, 12 bp, Artificial Sequence
  index sequence
tgactaccgtaa

SEQ ID NO: 400 - DNA, 12 bp, Artificial Sequence
  index sequence
ctttcatgtctc

SEQ ID NO: 401 - DNA, 12 bp, Artificial Sequence
  index sequence
gcacctagcggc

SEQ ID NO: 402 - DNA, 12 bp, Artificial Sequence
  index sequence
ctccgtctagag

SEQ ID NO: 403 - DNA, 12 bp, Artificial Sequence
  index sequence
gtcgctagccag

SEQ ID NO: 404 - DNA, 12 bp, Artificial Sequence
  index sequence
ttcggttgtata

SEQ ID NO: 405 - DNA, 12 bp, Artificial Sequence
  index sequence
gcggtatcatca

SEQ ID NO: 406 - DNA, 12 bp, Artificial Sequence
  index sequence
taaagcgtacgc

SEQ ID NO: 407 - DNA, 12 bp, Artificial Sequence
  index sequence
ttcttacgcaag

SEQ ID NO: 408 - DNA, 12 bp, Artificial Sequence
  index sequence
acgcgcggacta

SEQ ID NO: 409 - DNA, 12 bp, Artificial Sequence
  index sequence
agctataagatc

SEQ ID NO: 410 - DNA, 12 bp, Artificial Sequence
  index sequence
gtaatggcaaca

SEQ ID NO: 411 - DNA, 12 bp, Artificial Sequence
  index sequence
tccatttgatgc

SEQ ID NO: 412 - DNA, 12 bp, Artificial Sequence
  index sequence
cagggatttcca

SEQ ID NO: 413 - DNA, 12 bp, Artificial Sequence
  index sequence
caatcaatggac

SEQ ID NO: 414 - DNA, 12 bp, Artificial Sequence
  index sequence
cgattctgattg

SEQ ID NO: 415 - DNA, 12 bp, Artificial Sequence
  index sequence
tgggtcttcgcc

SEQ ID NO: 416 - DNA, 12 bp, Artificial Sequence
  index sequence
gtcgtcgaacgc

SEQ ID NO: 417 - DNA, 12 bp, Artificial Sequence
  index sequence
gaagtgccccca

SEQ ID NO: 418 - DNA, 12 bp, Artificial Sequence
  index sequence
gccgggaataag

SEQ ID NO: 419 - DNA, 12 bp, Artificial Sequence
  index sequence
actttggaatag

SEQ ID NO: 420 - DNA, 12 bp, Artificial Sequence
  index sequence
ttctggtcccag

SEQ ID NO: 421 - DNA, 12 bp, Artificial Sequence
  index sequence
aacttaatttct

SEQ ID NO: 422 - DNA, 12 bp, Artificial Sequence
  index sequence
tcgaagtgctgt

SEQ ID NO: 423 - DNA, 12 bp, Artificial Sequence
  index sequence
tcgcaacacgct

SEQ ID NO: 424 - DNA, 12 bp, Artificial Sequence
  index sequence
gtatcttgtcac

SEQ ID NO: 425 - DNA, 12 bp, Artificial Sequence
  index sequence
catgaagaggcg

SEQ ID NO: 426 - DNA, 12 bp, Artificial Sequence
  index sequence
tacgagctggtt

SEQ ID NO: 427 - DNA, 12 bp, Artificial Sequence
  index sequence
cccttactgtga

SEQ ID NO: 428 - DNA, 12 bp, Artificial Sequence
  index sequence
tccggtgcattt

SEQ ID NO: 429 - DNA, 12 bp, Artificial Sequence
  index sequence
gccaaggtgcta

SEQ ID NO: 430 - DNA, 12 bp, Artificial Sequence
  index sequence
cttccgcaaact

SEQ ID NO: 431 - DNA, 12 bp, Artificial Sequence
  index sequence
cggaagggaacc

SEQ ID NO: 432 - DNA, 12 bp, Artificial Sequence
  index sequence
cgccgcgttaag

SEQ ID NO: 433 - DNA, 12 bp, Artificial Sequence
  index sequence
ccttctagttat

SEQ ID NO: 434 - DNA, 12 bp, Artificial Sequence
  index sequence
ttgtgaaacatt

SEQ ID NO: 435 - DNA, 12 bp, Artificial Sequence
  index sequence
ccagtcctgact

SEQ ID NO: 436 - DNA, 12 bp, Artificial Sequence
  index sequence
tccttaacccgt

SEQ ID NO: 437 - DNA, 12 bp, Artificial Sequence
  index sequence
tgaaacgcgcaa

SEQ ID NO: 438 - DNA, 12 bp, Artificial Sequence
  index sequence
cgtccttgatcc

SEQ ID NO: 439 - DNA, 12 bp, Artificial Sequence
  index sequence
actggcagcggg

SEQ ID NO: 440 - DNA, 12 bp, Artificial Sequence
  index sequence
cgttcacagccg

SEQ ID NO: 441 - DNA, 12 bp, Artificial Sequence
  index sequence
tgaatcctcgag

SEQ ID NO: 442 - DNA, 12 bp, Artificial Sequence
  index sequence
tgcgtcgcctta

SEQ ID NO: 443 - DNA, 12 bp, Artificial Sequence
  index sequence
tctgaccagaaa

SEQ ID NO: 444 - DNA, 12 bp, Artificial Sequence
  index sequence
tattccgtccaa

SEQ ID NO: 445 - DNA, 12 bp, Artificial Sequence
  index sequence
agatttcgctac

SEQ ID NO: 446 - DNA, 12 bp, Artificial Sequence
  index sequence
caatgctcaatt

SEQ ID NO: 447 - DNA, 12 bp, Artificial Sequence
  index sequence
tctttgccccat

SEQ ID NO: 448 - DNA, 12 bp, Artificial Sequence
  index sequence
ctatatacgcgg

SEQ ID NO: 449 - DNA, 12 bp, Artificial Sequence
  index sequence
ccttagcaaatc

SEQ ID NO: 450 - DNA, 12 bp, Artificial Sequence
  index sequence
tcgtactaatcg

SEQ ID NO: 451 - DNA, 12 bp, Artificial Sequence
  index sequence
gagcccctgctc

SEQ ID NO: 452 - DNA, 12 bp, Artificial Sequence
  index sequence
gttgctgtccac

SEQ ID NO: 453 - DNA, 12 bp, Artificial Sequence
  index sequence
cgtgggaatgtc

SEQ ID NO: 454 - DNA, 12 bp, Artificial Sequence
  index sequence
atcatggatagg

SEQ ID NO: 455 - DNA, 12 bp, Artificial Sequence
  index sequence
gacttagcccct

SEQ ID NO: 456 - DNA, 12 bp, Artificial Sequence
  index sequence
tcgtgtatgact

SEQ ID NO: 457 - DNA, 12 bp, Artificial Sequence
  index sequence
aatgtcatgcat

SEQ ID NO: 458 - DNA, 12 bp, Artificial Sequence
  index sequence
ccccgttcttat

SEQ ID NO: 459 - DNA, 12 bp, Artificial Sequence
  index sequence
tgggatatttac

SEQ ID NO: 460 - DNA, 12 bp, Artificial Sequence
  index sequence
tccctgtcatcg

SEQ ID NO: 461 - DNA, 12 bp, Artificial Sequence
  index sequence
ttaaagtagagt

SEQ ID NO: 462 - DNA, 12 bp, Artificial Sequence
  index sequence
gcacttgtatcc

SEQ ID NO: 463 - DNA, 12 bp, Artificial Sequence
  index sequence
ctagttgcgcat

SEQ ID NO: 464 - DNA, 12 bp, Artificial Sequence
  index sequence
gttctttgctga

SEQ ID NO: 465 - DNA, 12 bp, Artificial Sequence
  index sequence
tatatttcttat

SEQ ID NO: 466 - DNA, 12 bp, Artificial Sequence
  index sequence
ctgaaacagggg

SEQ ID NO: 467 - DNA, 12 bp, Artificial Sequence
  index sequence
gagggttgctaa

SEQ ID NO: 468 - DNA, 12 bp, Artificial Sequence
  index sequence
ctagggtgccag

SEQ ID NO: 469 - DNA, 12 bp, Artificial Sequence
  index sequence
cggtcattcgcg

SEQ ID NO: 470 - DNA, 12 bp, Artificial Sequence
  index sequence
gatgtattggtt

SEQ ID NO: 471 - DNA, 12 bp, Artificial Sequence
  index sequence
cctagagtaggt

SEQ ID NO: 472 - DNA, 12 bp, Artificial Sequence
  index sequence
caagaaaccacg

SEQ ID NO: 473 - DNA, 12 bp, Artificial Sequence
  index sequence
tgtggaaggaat

SEQ ID NO: 474 - DNA, 12 bp, Artificial Sequence
  index sequence
tgcgtatggttg

SEQ ID NO: 475 - DNA, 12 bp, Artificial Sequence
  index sequence
acgggtgatcac

SEQ ID NO: 476 - DNA, 12 bp, Artificial Sequence
  index sequence
accgttggtgac

SEQ ID NO: 477 - DNA, 12 bp, Artificial Sequence
  index sequence
atcagctgataa

SEQ ID NO: 478 - DNA, 12 bp, Artificial Sequence
  index sequence
gctatcggctgg

SEQ ID NO: 479 - DNA, 12 bp, Artificial Sequence
  index sequence
agacagctaaag

SEQ ID NO: 480 - DNA, 12 bp, Artificial Sequence
  index sequence
gaggtccacata

SEQ ID NO: 481 - DNA, 12 bp, Artificial Sequence
  index sequence
gtcctgcactgg

SEQ ID NO: 482 - DNA, 12 bp, Artificial Sequence
  index sequence
cttgagccttaa

SEQ ID NO: 483 - DNA, 12 bp, Artificial Sequence
  index sequence
acacacactagc

SEQ ID NO: 484 - DNA, 12 bp, Artificial Sequence
  index sequence
agggactccctt

SEQ ID NO: 485 - DNA, 12 bp, Artificial Sequence
  index sequence
aaggacaatatt

SEQ ID NO: 486 - DNA, 12 bp, Artificial Sequence
  index sequence
atacatatatat

SEQ ID NO: 487 - DNA, 12 bp, Artificial Sequence
  index sequence
cctatgcttcct

SEQ ID NO: 488 - DNA, 12 bp, Artificial Sequence
  index sequence
cggctggactgc

SEQ ID NO: 489 - DNA, 12 bp, Artificial Sequence
  index sequence
accctcataagg

SEQ ID NO: 490 - DNA, 12 bp, Artificial Sequence
  index sequence
tagtagccgcac

SEQ ID NO: 491 - DNA, 12 bp, Artificial Sequence
  index sequence
gatcatctggaa

SEQ ID NO: 492 - DNA, 12 bp, Artificial Sequence
  index sequence
gagttataaatt

SEQ ID NO: 493 - DNA, 12 bp, Artificial Sequence
  index sequence
gtgtccttacat

SEQ ID NO: 494 - DNA, 12 bp, Artificial Sequence
  index sequence
cgaatgcagaaa

SEQ ID NO: 495 - DNA, 12 bp, Artificial Sequence
  index sequence
cgagagattgat

SEQ ID NO: 496 - DNA, 12 bp, Artificial Sequence
  index sequence
accggctcgacc

SEQ ID NO: 497 - DNA, 12 bp, Artificial Sequence
  index sequence
cgtcttctgaaa

SEQ ID NO: 498 - DNA, 12 bp, Artificial Sequence
  index sequence
cgacacattcac

SEQ ID NO: 499 - DNA, 12 bp, Artificial Sequence
  index sequence
cgcctgtagcac

SEQ ID NO: 500 - DNA, 12 bp, Artificial Sequence
  index sequence
ccgtccacgatt

SEQ ID NO: 501 - DNA, 12 bp, Artificial Sequence
  index sequence
tcgcatatgcat

SEQ ID NO: 502 - DNA, 12 bp, Artificial Sequence
  index sequence
ctcgcagctaaa

SEQ ID NO: 503 - DNA, 12 bp, Artificial Sequence
  index sequence
tactgaagccat

SEQ ID NO: 504 - DNA, 12 bp, Artificial Sequence
  index sequence
agtagcctctgg

SEQ ID NO: 505 - DNA, 12 bp, Artificial Sequence
  index sequence
ctgcaaacgctg

SEQ ID NO: 506 - DNA, 12 bp, Artificial Sequence
  index sequence
ctttggaagctt

SEQ ID NO: 507 - DNA, 12 bp, Artificial Sequence
  index sequence
cgtggagaccga

SEQ ID NO: 508 - DNA, 12 bp, Artificial Sequence
  index sequence
agaattttcggg

SEQ ID NO: 509 - DNA, 12 bp, Artificial Sequence
  index sequence
ataggtgctagt

SEQ ID NO: 510 - DNA, 12 bp, Artificial Sequence
  index sequence
aagtgtgatgcc

SEQ ID NO: 511 - DNA, 12 bp, Artificial Sequence
  index sequence
ctaatgtgaatc

SEQ ID NO: 512 - DNA, 12 bp, Artificial Sequence
  index sequence
tatcctatgcag

SEQ ID NO: 513 - DNA, 12 bp, Artificial Sequence
  index sequence
cgtggctccgtt

SEQ ID NO: 514 - DNA, 12 bp, Artificial Sequence
  index sequence
tgaaatacccaa

SEQ ID NO: 515 - DNA, 12 bp, Artificial Sequence
  index sequence
ataaaatgtgca

SEQ ID NO: 516 - DNA, 12 bp, Artificial Sequence
  index sequence
gtctgaggtcga

SEQ ID NO: 517 - DNA, 12 bp, Artificial Sequence
  index sequence
aacatcactatt

SEQ ID NO: 518 - DNA, 12 bp, Artificial Sequence
  index sequence
atcccattattg

SEQ ID NO: 519 - DNA, 12 bp, Artificial Sequence
  index sequence
gacgctctggtc

SEQ ID NO: 520 - DNA, 12 bp, Artificial Sequence
  index sequence
tatgattgcggt

SEQ ID NO: 521 - DNA, 12 bp, Artificial Sequence
  index sequence
gccctgtgccgg

SEQ ID NO: 522 - DNA, 12 bp, Artificial Sequence
  index sequence
acccagatgcgg

SEQ ID NO: 523 - DNA, 12 bp, Artificial Sequence
  index sequence
gatcatttgggg

SEQ ID NO: 524 - DNA, 12 bp, Artificial Sequence
  index sequence
cgcccttggact

SEQ ID NO: 525 - DNA, 12 bp, Artificial Sequence
  index sequence
atgaaccacagc

SEQ ID NO: 526 - DNA, 12 bp, Artificial Sequence
  index sequence
aaccctaattag

SEQ ID NO: 527 - DNA, 12 bp, Artificial Sequence
  index sequence
agaaaccctcta

SEQ ID NO: 528 - DNA, 12 bp, Artificial Sequence
  index sequence
tttctagttcct

SEQ ID NO: 529 - DNA, 12 bp, Artificial Sequence
  index sequence
cagtaccagtaa

SEQ ID NO: 530 - DNA, 12 bp, Artificial Sequence
  index sequence
tacggtcccatt

SEQ ID NO: 531 - DNA, 12 bp, Artificial Sequence
  index sequence
cgcgtcttcgcg

SEQ ID NO: 532 - DNA, 12 bp, Artificial Sequence
  index sequence
tcactggaacat

SEQ ID NO: 533 - DNA, 12 bp, Artificial Sequence
  index sequence
gacggttatagt

SEQ ID NO: 534 - DNA, 12 bp, Artificial Sequence
  index sequence
agctgctccagg

SEQ ID NO: 535 - DNA, 12 bp, Artificial Sequence
  index sequence
cgttatcaggca

SEQ ID NO: 536 - DNA, 12 bp, Artificial Sequence
  index sequence
tatacgcttact

SEQ ID NO: 537 - DNA, 12 bp, Artificial Sequence
  index sequence
catgtaaagatc

SEQ ID NO: 538 - DNA, 12 bp, Artificial Sequence
  index sequence
ctgcaggtgcga

SEQ ID NO: 539 - DNA, 12 bp, Artificial Sequence
  index sequence
gcaagtgagacc

SEQ ID NO: 540 - DNA, 12 bp, Artificial Sequence
  index sequence
tcatagtgatgt

SEQ ID NO: 541 - DNA, 12 bp, Artificial Sequence
  index sequence
gttactcctaca

SEQ ID NO: 542 - DNA, 12 bp, Artificial Sequence
  index sequence
cgcgccgagttc

SEQ ID NO: 543 - DNA, 12 bp, Artificial Sequence
  index sequence
cggcactaggca

SEQ ID NO: 544 - DNA, 12 bp, Artificial Sequence
  index sequence
tgagttccatat

SEQ ID NO: 545 - DNA, 12 bp, Artificial Sequence
  index sequence
ccattgtccctc

SEQ ID NO: 546 - DNA, 12 bp, Artificial Sequence
  index sequence
tctaatcatact

SEQ ID NO: 547 - DNA, 12 bp, Artificial Sequence
  index sequence
aacagcgacatg

SEQ ID NO: 548 - DNA, 12 bp, Artificial Sequence
  index sequence
gagttagctgcc

SEQ ID NO: 549 - DNA, 12 bp, Artificial Sequence
  index sequence
ttcgatctattg

SEQ ID NO: 550 - DNA, 12 bp, Artificial Sequence
  index sequence
cggtaatggggc

SEQ ID NO: 551 - DNA, 12 bp, Artificial Sequence
  index sequence
cattagtaacgt

SEQ ID NO: 552 - DNA, 12 bp, Artificial Sequence
  index sequence
tcgtgattatcc

SEQ ID NO: 553 - DNA, 12 bp, Artificial Sequence
  index sequence
gaaggcggtatg

SEQ ID NO: 554 - DNA, 12 bp, Artificial Sequence
  index sequence
gttagctacgtc

SEQ ID NO: 555 - DNA, 12 bp, Artificial Sequence
  index sequence
aacgccgttctt

SEQ ID NO: 556 - DNA, 12 bp, Artificial Sequence
  index sequence
actcgggcgggg

SEQ ID NO: 557 - DNA, 12 bp, Artificial Sequence
  index sequence
acggagagccgc

SEQ ID NO: 558 - DNA, 12 bp, Artificial Sequence
  index sequence
aaagctcgtcac

SEQ ID NO: 559 - DNA, 12 bp, Artificial Sequence
  index sequence
cgaaagagtagt

SEQ ID NO: 560 - DNA, 12 bp, Artificial Sequence
  index sequence
tggaactcagtc

SEQ ID NO: 561 - DNA, 12 bp, Artificial Sequence
  index sequence
ccgaggacgcgg

SEQ ID NO: 562 - DNA, 12 bp, Artificial Sequence
  index sequence
tcagacgtcacc

SEQ ID NO: 563 - DNA, 12 bp, Artificial Sequence
  index sequence
tatgtccttgac

SEQ ID NO: 564 - DNA, 12 bp, Artificial Sequence
  index sequence
tcaacttagacg

SEQ ID NO: 565 - DNA, 12 bp, Artificial Sequence
  index sequence
agaccgaaatag

SEQ ID NO: 566 - DNA, 12 bp, Artificial Sequence
  index sequence
acagagctggga

SEQ ID NO: 567 - DNA, 12 bp, Artificial Sequence
  index sequence
acacaccgggcg

SEQ ID NO: 568 - DNA, 12 bp, Artificial Sequence
  index sequence
ttcgtgttcccc

SEQ ID NO: 569 - DNA, 12 bp, Artificial Sequence
  index sequence
tcggggcactac

SEQ ID NO: 570 - DNA, 12 bp, Artificial Sequence
  index sequence
gcccgctagaag

SEQ ID NO: 571 - DNA, 12 bp, Artificial Sequence
  index sequence
gccagcgcctgt

SEQ ID NO: 572 - DNA, 12 bp, Artificial Sequence
  index sequence
gaataataagtg

SEQ ID NO: 573 - DNA, 12 bp, Artificial Sequence
  index sequence
atgctgtgcgcg

SEQ ID NO: 574 - DNA, 12 bp, Artificial Sequence
  index sequence
cttgctaccgat

SEQ ID NO: 575 - DNA, 12 bp, Artificial Sequence
  index sequence
cgcagggacacc

SEQ ID NO: 576 - DNA, 12 bp, Artificial Sequence
  index sequence
aaatgattcagc

SEQ ID NO: 577 - DNA, 12 bp, Artificial Sequence
  index sequence
ttcctgagtgct

SEQ ID NO: 578 - DNA, 12 bp, Artificial Sequence
  index sequence
gtgatcctgggc

SEQ ID NO: 579 - DNA, 12 bp, Artificial Sequence
  index sequence
attccacactcc

SEQ ID NO: 580 - DNA, 12 bp, Artificial Sequence
  index sequence
cccccaggacgg

SEQ ID NO: 581 - DNA, 12 bp, Artificial Sequence
  index sequence
tgtttgcgtagg

SEQ ID NO: 582 - DNA, 12 bp, Artificial Sequence
  index sequence
tgaaagcacggt

SEQ ID NO: 583 - DNA, 12 bp, Artificial Sequence
  index sequence
ccagcctatgtc

SEQ ID NO: 584 - DNA, 12 bp, Artificial Sequence
  index sequence
gtactaagtttt

SEQ ID NO: 585 - DNA, 12 bp, Artificial Sequence
  index sequence
ctccatataata

SEQ ID NO: 586 - DNA, 12 bp, Artificial Sequence
  index sequence
tcgcctcaggtt

SEQ ID NO: 587 - DNA, 12 bp, Artificial Sequence
  index sequence
cagttttgctta

SEQ ID NO: 588 - DNA, 12 bp, Artificial Sequence
  index sequence
agcaatgccagg

SEQ ID NO: 589 - DNA, 12 bp, Artificial Sequence
  index sequence
cgtgtgcaaggt

SEQ ID NO: 590 - DNA, 12 bp, Artificial Sequence
  index sequence
ttctccgaagta

SEQ ID NO: 591 - DNA, 12 bp, Artificial Sequence
  index sequence
tcttgccataac

SEQ ID NO: 592 - DNA, 12 bp, Artificial Sequence
  index sequence
acgttaatccaa

SEQ ID NO: 593 - DNA, 12 bp, Artificial Sequence
  index sequence
cacttaccgtga

SEQ ID NO: 594 - DNA, 12 bp, Artificial Sequence
  index sequence
gagcagatagtc

SEQ ID NO: 595 - DNA, 12 bp, Artificial Sequence
  index sequence
agtgctttcccg

SEQ ID NO: 596 - DNA, 12 bp, Artificial Sequence
  index sequence
caatcacgcaat

SEQ ID NO: 597 - DNA, 12 bp, Artificial Sequence
  index sequence
gtttcttacgtg

SEQ ID NO: 598 - DNA, 12 bp, Artificial Sequence
  index sequence
gatacaaatatt

SEQ ID NO: 599 - DNA, 12 bp, Artificial Sequence
  index sequence
caatgctgtctt

SEQ ID NO: 600 - DNA, 12 bp, Artificial Sequence
  index sequence
cgttctgtgacg

SEQ ID NO: 601 - DNA, 12 bp, Artificial Sequence
  index sequence
taggatacaccg

SEQ ID NO: 602 - DNA, 12 bp, Artificial Sequence
  index sequence
gatgactcaccg

SEQ ID NO: 603 - DNA, 12 bp, Artificial Sequence
  index sequence
gaaaacactgct

SEQ ID NO: 604 - DNA, 12 bp, Artificial Sequence
  index sequence
cccgaatctaca

SEQ ID NO: 605 - DNA, 12 bp, Artificial Sequence
  index sequence
atctgtttttga

SEQ ID NO: 606 - DNA, 12 bp, Artificial Sequence
  index sequence
acagggtacgcc

SEQ ID NO: 607 - DNA, 12 bp, Artificial Sequence
  index sequence
gagtcggaccgc

SEQ ID NO: 608 - DNA, 12 bp, Artificial Sequence
  index sequence
tgtagaccagga

SEQ ID NO: 609 - DNA, 12 bp, Artificial Sequence
  index sequence
ctatacttctgg

SEQ ID NO: 610 - DNA, 12 bp, Artificial Sequence
  index sequence
gcgctacgtacg

SEQ ID NO: 611 - DNA, 12 bp, Artificial Sequence
  index sequence
ttagccaagcgc

SEQ ID NO: 612 - DNA, 12 bp, Artificial Sequence
  index sequence
atacataagaaa

SEQ ID NO: 613 - DNA, 12 bp, Artificial Sequence
  index sequence
tttgacccgaag

SEQ ID NO: 614 - DNA, 12 bp, Artificial Sequence
  index sequence
attgtccagcgt

SEQ ID NO: 615 - DNA, 12 bp, Artificial Sequence
  index sequence
gcgtgtatgcgg

SEQ ID NO: 616 - DNA, 12 bp, Artificial Sequence
  index sequence
caggagaacggg

SEQ ID NO: 617 - DNA, 12 bp, Artificial Sequence
  index sequence
gtccgacagtct

SEQ ID NO: 618 - DNA, 12 bp, Artificial Sequence
  index sequence
ccgtatttgtag

SEQ ID NO: 619 - DNA, 12 bp, Artificial Sequence
  index sequence
gcattacctagc

SEQ ID NO: 620 - DNA, 12 bp, Artificial Sequence
  index sequence
tatcgcacccgt

SEQ ID NO: 621 - DNA, 12 bp, Artificial Sequence
  index sequence
gctgagataatt

SEQ ID NO: 622 - DNA, 12 bp, Artificial Sequence
  index sequence
gtcataaacctg

SEQ ID NO: 623 - DNA, 12 bp, Artificial Sequence
  index sequence
tcgagcctctat

SEQ ID NO: 624 - DNA, 12 bp, Artificial Sequence
  index sequence
gacttgagcctt

SEQ ID NO: 625 - DNA, 12 bp, Artificial Sequence
  index sequence
ctggatggatac

SEQ ID NO: 626 - DNA, 12 bp, Artificial Sequence
  index sequence
tctacctcaaag

SEQ ID NO: 627 - DNA, 12 bp, Artificial Sequence
  index sequence
tactcccggaac

SEQ ID NO: 628 - DNA, 12 bp, Artificial Sequence
  index sequence
tgtgaaatctcc

SEQ ID NO: 629 - DNA, 12 bp, Artificial Sequence
  index sequence
cggaccgccagt

SEQ ID NO: 630 - DNA, 12 bp, Artificial Sequence
  index sequence
gtgaggaagcgt

SEQ ID NO: 631 - DNA, 12 bp, Artificial Sequence
  index sequence
gaggcgacaaac

SEQ ID NO: 632 - DNA, 12 bp, Artificial Sequence
  index sequence
agataggtgggc

SEQ ID NO: 633 - DNA, 12 bp, Artificial Sequence
  index sequence
caaatcgctaga

SEQ ID NO: 634 - DNA, 12 bp, Artificial Sequence
  index sequence
acgccagcctaa

SEQ ID NO: 635 - DNA, 12 bp, Artificial Sequence
  index sequence
aagacctgccat

SEQ ID NO: 636 - DNA, 12 bp, Artificial Sequence
  index sequence
tgcgcggggtta

SEQ ID NO: 637 - DNA, 12 bp, Artificial Sequence
  index sequence
actcattctttg

SEQ ID NO: 638 - DNA, 12 bp, Artificial Sequence
  index sequence
actagcagtcag

SEQ ID NO: 639 - DNA, 12 bp, Artificial Sequence
  index sequence
gaactatctcgc

SEQ ID NO: 640 - DNA, 12 bp, Artificial Sequence
  index sequence
gaatatgccatc

SEQ ID NO: 641 - DNA, 12 bp, Artificial Sequence
  index sequence
aaacggacgatt

SEQ ID NO: 642 - DNA, 12 bp, Artificial Sequence
  index sequence
tcgaaaggggac

SEQ ID NO: 643 - DNA, 12 bp, Artificial Sequence
  index sequence
acagtcaacgta

SEQ ID NO: 644 - DNA, 12 bp, Artificial Sequence
  index sequence
cctaaggagaca

SEQ ID NO: 645 - DNA, 12 bp, Artificial Sequence
  index sequence
aatatagcactt

SEQ ID NO: 646 - DNA, 12 bp, Artificial Sequence
  index sequence
catgagctagta

SEQ ID NO: 647 - DNA, 12 bp, Artificial Sequence
  index sequence
gtaaccataccc

SEQ ID NO: 648 - DNA, 12 bp, Artificial Sequence
  index sequence
tttattaataga

SEQ ID NO: 649 - DNA, 12 bp, Artificial Sequence
  index sequence
tcgaagttgtca

SEQ ID NO: 650 - DNA, 12 bp, Artificial Sequence
  index sequence
gcagctaataca

SEQ ID NO: 651 - DNA, 12 bp, Artificial Sequence
  index sequence
gtgattgaccca

SEQ ID NO: 652 - DNA, 12 bp, Artificial Sequence
  index sequence
acgtgcggtcat

SEQ ID NO: 653 - DNA, 12 bp, Artificial Sequence
  index sequence
tcgtttcgggtg

SEQ ID NO: 654 - DNA, 12 bp, Artificial Sequence
  index sequence
ttttagggctgg

SEQ ID NO: 655 - DNA, 12 bp, Artificial Sequence
  index sequence
gcttcactgcgc

SEQ ID NO: 656 - DNA, 12 bp, Artificial Sequence
  index sequence
ttaccaggtccg

SEQ ID NO: 657 - DNA, 12 bp, Artificial Sequence
  index sequence
ccggtcgctgag

SEQ ID NO: 658 - DNA, 12 bp, Artificial Sequence
  index sequence
ttacagcctgat

SEQ ID NO: 659 - DNA, 12 bp, Artificial Sequence
  index sequence
cttaaattggtc

SEQ ID NO: 660 - DNA, 12 bp, Artificial Sequence
  index sequence
cgataagctgaa

SEQ ID NO: 661 - DNA, 12 bp, Artificial Sequence
  index sequence
agaccatcgccg

SEQ ID NO: 662 - DNA, 12 bp, Artificial Sequence
  index sequence
tctggttcaacg

SEQ ID NO: 663 - DNA, 12 bp, Artificial Sequence
  index sequence
gatcagcgcgcg

SEQ ID NO: 664 - DNA, 12 bp, Artificial Sequence
  index sequence
tggaggaggagc

SEQ ID NO: 665 - DNA, 12 bp, Artificial Sequence
  index sequence
cgctggaccaaa

SEQ ID NO: 666 - DNA, 12 bp, Artificial Sequence
  index sequence
cgtccaacacga

SEQ ID NO: 667 - DNA, 12 bp, Artificial Sequence
  index sequence
aattttgtcaaa

SEQ ID NO: 668 - DNA, 12 bp, Artificial Sequence
  index sequence
ctccgccgtgaa

SEQ ID NO: 669 - DNA, 12 bp, Artificial Sequence
  index sequence
cctaggcgtcgc

SEQ ID NO: 670 - DNA, 12 bp, Artificial Sequence
  index sequence
gacgtccgatgt

SEQ ID NO: 671 - DNA, 12 bp, Artificial Sequence
  index sequence
agaggacagctc

SEQ ID NO: 672 - DNA, 12 bp, Artificial Sequence
  index sequence
atgacgatcatt

SEQ ID NO: 673 - DNA, 12 bp, Artificial Sequence
  index sequence
cacgggggtgta

SEQ ID NO: 674 - DNA, 12 bp, Artificial Sequence
  index sequence
gctaaccgcggg

SEQ ID NO: 675 - DNA, 12 bp, Artificial Sequence
  index sequence
gcacgtagcgcg

SEQ ID NO: 676 - DNA, 12 bp, Artificial Sequence
  index sequence
gttggcgccctc

SEQ ID NO: 677 - DNA, 12 bp, Artificial Sequence
  index sequence
tacatatcggct

SEQ ID NO: 678 - DNA, 12 bp, Artificial Sequence
  index sequence
ttcctcccagtc

SEQ ID NO: 679 - DNA, 12 bp, Artificial Sequence
  index sequence
ttgctcttagac

SEQ ID NO: 680 - DNA, 12 bp, Artificial Sequence
  index sequence
agttggatagag

SEQ ID NO: 681 - DNA, 12 bp, Artificial Sequence
  index sequence
agtatgtattac

SEQ ID NO: 682 - DNA, 12 bp, Artificial Sequence
  index sequence
ccacgtgtacaa

SEQ ID NO: 683 - DNA, 12 bp, Artificial Sequence
  index sequence
gagcttccctac

SEQ ID NO: 684 - DNA, 12 bp, Artificial Sequence
  index sequence
aggcgaagcaag

SEQ ID NO: 685 - DNA, 12 bp, Artificial Sequence
  index sequence
gtctcgttgagc

SEQ ID NO: 686 - DNA, 12 bp, Artificial Sequence
  index sequence
agcgactagggt

SEQ ID NO: 687 - DNA, 12 bp, Artificial Sequence
  index sequence
tgcatcaagtcc

SEQ ID NO: 688 - DNA, 12 bp, Artificial Sequence
  index sequence
atttactgtata

SEQ ID NO: 689 - DNA, 12 bp, Artificial Sequence
  index sequence
gacaatcgagga

SEQ ID NO: 690 - DNA, 12 bp, Artificial Sequence
  index sequence
ataagtatcgcg

SEQ ID NO: 691 - DNA, 12 bp, Artificial Sequence
  index sequence
gtagatcgaacg

SEQ ID NO: 692 - DNA, 12 bp, Artificial Sequence
  index sequence
ttaggttgtctc

SEQ ID NO: 693 - DNA, 12 bp, Artificial Sequence
  index sequence
gaggtctactac

SEQ ID NO: 694 - DNA, 12 bp, Artificial Sequence
  index sequence
tcccgagtcaga

SEQ ID NO: 695 - DNA, 12 bp, Artificial Sequence
  index sequence
ttattcagaccg

SEQ ID NO: 696 - DNA, 12 bp, Artificial Sequence
  index sequence
cagagaggcatc

SEQ ID NO: 697 - DNA, 12 bp, Artificial Sequence
  index sequence
cgatctccgcta

SEQ ID NO: 698 - DNA, 12 bp, Artificial Sequence
  index sequence
gtcctggaccac

SEQ ID NO: 699 - DNA, 12 bp, Artificial Sequence
  index sequence
taactttgctga

SEQ ID NO: 700 - DNA, 12 bp, Artificial Sequence
  index sequence
acgggctttaac

SEQ ID NO: 701 - DNA, 12 bp, Artificial Sequence
  index sequence
acctacctggca

SEQ ID NO: 702 - DNA, 12 bp, Artificial Sequence
  index sequence
agcttatgcttg

SEQ ID NO: 703 - DNA, 12 bp, Artificial Sequence
  index sequence
tgggtattagaa

SEQ ID NO: 704 - DNA, 12 bp, Artificial Sequence
  index sequence
gtagtagccaga

SEQ ID NO: 705 - DNA, 12 bp, Artificial Sequence
  index sequence
gccgtgaaaaac

SEQ ID NO: 706 - DNA, 12 bp, Artificial Sequence
  index sequence
gaagggcctccg

SEQ ID NO: 707 - DNA, 12 bp, Artificial Sequence
  index sequence
catttggcctcg

SEQ ID NO: 708 - DNA, 12 bp, Artificial Sequence
  index sequence
ttatggtaaacg

SEQ ID NO: 709 - DNA, 12 bp, Artificial Sequence
  index sequence
ccattcctttat

SEQ ID NO: 710 - DNA, 12 bp, Artificial Sequence
  index sequence
tagccgtgatgt

SEQ ID NO: 711 - DNA, 12 bp, Artificial Sequence
  index sequence
tagaccacagat

SEQ ID NO: 712 - DNA, 12 bp, Artificial Sequence
  index sequence
gtctattgtaca

SEQ ID NO: 713 - DNA, 12 bp, Artificial Sequence
  index sequence
actgccgcggag

SEQ ID NO: 714 - DNA, 12 bp, Artificial Sequence
  index sequence
tcagcgatggtt

SEQ ID NO: 715 - DNA, 12 bp, Artificial Sequence
  index sequence
aaattcatgtgc

SEQ ID NO: 716 - DNA, 12 bp, Artificial Sequence
  index sequence
taaggtgacttt

SEQ ID NO: 717 - DNA, 12 bp, Artificial Sequence
  index sequence
gaaccggtgatc

SEQ ID NO: 718 - DNA, 12 bp, Artificial Sequence
  index sequence
attaagacccat

SEQ ID NO: 719 - DNA, 12 bp, Artificial Sequence
  index sequence
aggccgggccaa

SEQ ID NO: 720 - DNA, 12 bp, Artificial Sequence
  index sequence
agaagagttccg

SEQ ID NO: 721 - DNA, 12 bp, Artificial Sequence
  index sequence
aattatcgttct

SEQ ID NO: 722 - DNA, 12 bp, Artificial Sequence
  index sequence
ttgtgcccactt

SEQ ID NO: 723 - DNA, 12 bp, Artificial Sequence
  index sequence
aacgtaatgcat

SEQ ID NO: 724 - DNA, 12 bp, Artificial Sequence
  index sequence
taattccaaagt

SEQ ID NO: 725 - DNA, 12 bp, Artificial Sequence
  index sequence
tgcccagagacc

SEQ ID NO: 726 - DNA, 12 bp, Artificial Sequence
  index sequence
agtaattgctaa

SEQ ID NO: 727 - DNA, 12 bp, Artificial Sequence
  index sequence
catggacgaggg

SEQ ID NO: 728 - DNA, 12 bp, Artificial Sequence
  index sequence
agttacacgaag

SEQ ID NO: 729 - DNA, 12 bp, Artificial Sequence
  index sequence
tgcctaatagcg

SEQ ID NO: 730 - DNA, 12 bp, Artificial Sequence
  index sequence
tgagtagaattc

SEQ ID NO: 731 - DNA, 12 bp, Artificial Sequence
  index sequence
tatgcaacgccc

SEQ ID NO: 732 - DNA, 12 bp, Artificial Sequence
  index sequence
tcttaagtaacc

SEQ ID NO: 733 - DNA, 12 bp, Artificial Sequence
  index sequence
cgctttagatca

SEQ ID NO: 734 - DNA, 12 bp, Artificial Sequence
  index sequence
acctgatacctt

SEQ ID NO: 735 - DNA, 12 bp, Artificial Sequence
  index sequence
tatttgaaaact

SEQ ID NO: 736 - DNA, 12 bp, Artificial Sequence
  index sequence
atctctcagagg

SEQ ID NO: 737 - DNA, 12 bp, Artificial Sequence
  index sequence
aattcgacccta

SEQ ID NO: 738 - DNA, 12 bp, Artificial Sequence
  index sequence
tagtcatcctag

SEQ ID NO: 739 - DNA, 12 bp, Artificial Sequence
  index sequence
gcgaaaatgata

SEQ ID NO: 740 - DNA, 12 bp, Artificial Sequence
  index sequence
gttgatgtaaca

SEQ ID NO: 741 - DNA, 12 bp, Artificial Sequence
  index sequence
agtgggcctgta

SEQ ID NO: 742 - DNA, 12 bp, Artificial Sequence
  index sequence
ctactggctcgg

SEQ ID NO: 743 - DNA, 12 bp, Artificial Sequence
  index sequence
gcattcgaaaat

SEQ ID NO: 744 - DNA, 12 bp, Artificial Sequence
  index sequence
tagtgtctgcat

SEQ ID NO: 745 - DNA, 12 bp, Artificial Sequence
  index sequence
cctgtactgact

SEQ ID NO: 746 - DNA, 12 bp, Artificial Sequence
  index sequence
aaaagttattct

SEQ ID NO: 747 - DNA, 12 bp, Artificial Sequence
  index sequence
tgggctctttca

SEQ ID NO: 748 - DNA, 12 bp, Artificial Sequence
  index sequence
taaatgtactag

SEQ ID NO: 749 - DNA, 12 bp, Artificial Sequence
  index sequence
ttcccgtcgcgt

SEQ ID NO: 750 - DNA, 12 bp, Artificial Sequence
  index sequence
gacattgtctaa

SEQ ID NO: 751 - DNA, 12 bp, Artificial Sequence
  index sequence
atcgttgagact

SEQ ID NO: 752 - DNA, 12 bp, Artificial Sequence
  index sequence
gttatttgatgc

SEQ ID NO: 753 - DNA, 12 bp, Artificial Sequence
  index sequence
tctctttattct

SEQ ID NO: 754 - DNA, 12 bp, Artificial Sequence
  index sequence
atgcccacgggg

SEQ ID NO: 755 - DNA, 12 bp, Artificial Sequence
  index sequence
gcgggttgatcc

SEQ ID NO: 756 - DNA, 12 bp, Artificial Sequence
  index sequence
atcgggtgaacg

SEQ ID NO: 757 - DNA, 12 bp, Artificial Sequence
  index sequence
aggtacttagag

SEQ ID NO: 758 - DNA, 12 bp, Artificial Sequence
  index sequence
gctgtcttggtt

SEQ ID NO: 759 - DNA, 12 bp, Artificial Sequence
  index sequence
aatcgcgtcggt

SEQ ID NO: 760 - DNA, 12 bp, Artificial Sequence
  index sequence
accgcccaacag

SEQ ID NO: 761 - DNA, 12 bp, Artificial Sequence
  index sequence
tgtggccggcct

SEQ ID NO: 762 - DNA, 12 bp, Artificial Sequence
  index sequence
tgagtctggttg

SEQ ID NO: 763 - DNA, 12 bp, Artificial Sequence
  index sequence
cagggtgctaca

SEQ ID NO: 764 - DNA, 12 bp, Artificial Sequence
  index sequence
caagttggtgca

SEQ ID NO: 765 - DNA, 12 bp, Artificial Sequence
  index sequence
ctacgatgctcc

SEQ ID NO: 766 - DNA, 12 bp, Artificial Sequence
  index sequence
gatctaggatgg

SEQ ID NO: 767 - DNA, 12 bp, Artificial Sequence
  index sequence
cgcacgatcccg

SEQ ID NO: 768 - DNA, 12 bp, Artificial Sequence
  index sequence
gcggtaacactc

SEQ ID NO: 769 - DNA, 12 bp, Artificial Sequence
  index sequence
gtaatgacatgg

SEQ ID NO: 770 - DNA, 12 bp, Artificial Sequence
  index sequence
attgcgaattcc

SEQ ID NO: 771 - DNA, 12 bp, Artificial Sequence
  index sequence
cacacacatcga

SEQ ID NO: 772 - DNA, 12 bp, Artificial Sequence
  index sequence
cgggcataaatt

SEQ ID NO: 773 - DNA, 12 bp, Artificial Sequence
  index sequence
ccggcacctctt

SEQ ID NO: 774 - DNA, 12 bp, Artificial Sequence
  index sequence
ctcactctctct

SEQ ID NO: 775 - DNA, 12 bp, Artificial Sequence
  index sequence
aatctgattaat

SEQ ID NO: 776 - DNA, 12 bp, Artificial Sequence
  index sequence
aggatggcatga

SEQ ID NO: 777 - DNA, 12 bp, Artificial Sequence
  index sequence
caaatactccgg

SEQ ID NO: 778 - DNA, 12 bp, Artificial Sequence
  index sequence
tcgtcgaagaca

SEQ ID NO: 779 - DNA, 12 bp, Artificial Sequence
  index sequence
gctactatggcc

SEQ ID NO: 780 - DNA, 12 bp, Artificial Sequence
  index sequence
gcgttctccctt

SEQ ID NO: 781 - DNA, 12 bp, Artificial Sequence
  index sequence
gtgtaattcact

SEQ ID NO: 782 - DNA, 12 bp, Artificial Sequence
  index sequence
agcctgacgccc

SEQ ID NO: 783 - DNA, 12 bp, Artificial Sequence
  index sequence
agcgcgcttgct

SEQ ID NO: 784 - DNA, 12 bp, Artificial Sequence
  index sequence
caaggatagcaa